European Patent Application EP 4 428 158 A1, published September 11, 2024. Title: LUNG CANCER TARGETING HUMAN ANTIBODIES AND THERAPEUTIC USES THEREOF. Applicant: Istituto Romagnolo per lo Studio dei Tumori "Dino Amadori" - IRST S.r.l. Application EP. The sequence listing filed with the application follows.

SEQUENCE LISTING (158 sequences)

SEQ ID NO: 1 - protein, 6 aa, synthetic construct
SSNWWS

SEQ ID NO: 2 - protein, 16 aa, synthetic construct
EIYHSGSTNYNPSLKS

SEQ ID NO: 3 - protein, 17 aa, synthetic construct
DKMVRGLIDYYYYGLDV

SEQ ID NO: 4 - protein, 7 aa, synthetic construct
ARLHFDY

SEQ ID NO: 5 - protein, 9 aa, synthetic construct
SYFDSGMDV

SEQ ID NO: 6 - protein, 12 aa, synthetic construct
GASQSVSSSYLA

SEQ ID NO: 7 - protein, 7 aa, synthetic construct
DASSRAT

SEQ ID NO: 8 - protein, 8 aa, synthetic construct
QQYGSSLT

SEQ ID NO: 9 - protein, 16 aa, synthetic construct
RSSQSLLHSNGYNYLD

SEQ ID NO: 10 - protein, 7 aa, synthetic construct
LGSNRAS

SEQ ID NO: 11 - protein, 11 aa, synthetic construct
MQALQTPPRFT

SEQ ID NO: 12 - protein, 11 aa, synthetic construct
RASQSVSSNLA

SEQ ID NO: 13 - protein, 7 aa, synthetic construct
QQYNKWP

SEQ ID NO: 14 - protein, 30 aa, synthetic construct
QVQLQESGPGLVKPPGTLSLTCAVSGGSIS

SEQ ID NO: 15 - protein, 14 aa, synthetic construct
WVRQPPGKGLEWIG

SEQ ID NO: 16 - protein, 32 aa, synthetic construct
RVTISVDTSKNQISLQLSSVTAADTAVYYCAR

SEQ ID NO: 17 - protein, 11 aa, synthetic construct
WGQGTTVTVSS

SEQ ID NO: 18 - protein, 23 aa, synthetic construct
EIVLTQSPATLSLSPGERATLSC

SEQ ID NO: 19 - protein, 15 aa, synthetic construct
WYQQKPGLAPRLLIY

SEQ ID NO: 20 - protein, 32 aa, synthetic construct
GIPDRFSGSGSGTDFTLTISRLEPEDFAVYYC

SEQ ID NO: 21 - protein, 10 aa, synthetic construct
FGQGTKVEIK

SEQ ID NO: 22 - protein, 32 aa, synthetic construct
RVTISVDKSKNHFSLYVSSVTAADTAVYYCAR

SEQ ID NO: 23 - protein, 11 aa, synthetic construct
WGQGTLVTVSS

SEQ ID NO: 24 - protein, 23 aa, synthetic construct
DIVMTQSPLSLPVTPGEPASISC

SEQ ID NO: 25 - protein, 15 aa, synthetic construct
WYLQKPGQSPQLLIY

SEQ ID NO: 26 - protein, 32 aa, synthetic construct
GVPDRFSGSGSGTDFTLKISRVEAEDVGVYYC

SEQ ID NO: 27 - protein, 10 aa, Synthetic construct
FGPGTKVDIK

SEQ ID NO: 28 - protein, 32 aa, synthetic construct
RVTISVDTSKNHFYLNLSSVTAADTALYYCAR

SEQ ID NO: 29 - protein, 23 aa, Synthetic construct
EIVMTQSPATLSVSPGERATLSC

SEQ ID NO: 30 - protein, 15 aa, synthetic construct
WYQQKLGQASRLLIY

SEQ ID NO: 31 - protein, 26 aa, synthetic construct
SGSGSGTEFTLTISSLQSEDFAVYYC

SEQ ID NO: 32 - protein, 25 aa, synthetic construct
QVQLQESGPGLVKPPGTLSLTCAVS

SEQ ID NO: 33 - protein, 29 aa, synthetic construct
QVQLQESGPGLVKPPGTLSLTCAVSGGSI

SEQ ID NO: 34 - protein, 8 aa, synthetic construct
GGSISSSN

SEQ ID NO: 35 - protein, 11 aa, synthetic construct
GGSISSSNWWS

SEQ ID NO: 36 - protein, 7 aa, synthetic construct
SSSNWWS

SEQ ID NO: 37 - protein, 9 aa, synthetic construct
GGSISSSNW

SEQ ID NO: 38 - protein, 19 aa, synthetic construct
WWSWVRQPPGKGLEWIGEI

SEQ ID NO: 39 - protein, 11 aa, synthetic construct
WVRQPPGKGLE

SEQ ID NO: 40 - protein, 17 aa, synthetic construct
WSWVRQPPGKGLEWIGE

SEQ ID NO: 41 - protein, 5 aa, synthetic construct
YHSGS

SEQ ID NO: 42 - protein, 9 aa, synthetic construct
EIYHSGSTN

SEQ ID NO: 43 - protein, 12 aa, synthetic construct
WIGEIYHSGSTN

SEQ ID NO: 44 - protein, 7 aa, synthetic construct
IYHSGST

SEQ ID NO: 45 - protein, 41 aa, synthetic construct
TNYNPSLKSRVTISVDTSKNQISLQLSSVTAADTAVYYCAR

SEQ ID NO: 46 - protein, 39 aa, synthetic construct
YNPSLKSRVTISVDTSKNQISLQLSSVTAADTAVYYCAR

SEQ ID NO: 47 - protein, 37 aa, synthetic construct
YNPSLKSRVTISVDTSKNQISLQLSSVTAADTAVYYC

SEQ ID NO: 48 - protein, 38 aa, synthetic construct
NYNPSLKSRVTISVDTSKNQISLQLSSVTAADTAVYYC

SEQ ID NO: 49 - protein, 18 aa, synthetic construct
ARDKMVRGLIDYYYYGLD

SEQ ID NO: 50 - protein, 19 aa, synthetic construct
ARDKMVRGLIDYYYYGLDV

SEQ ID NO: 51 - protein, 12 aa, synthetic construct
VWGQGTTVTVSS

SEQ ID NO: 52 - protein, 29 aa, synthetic construct
EIVLTQSPATLSLSPGERATLSCGASQSV

SEQ ID NO: 53 - protein, 26 aa, synthetic construct
EIVLTQSPATLSLSPGERATLSCGAS

SEQ ID NO: 54 - protein, 8 aa, synthetic construct
SSSYLAWY

SEQ ID NO: 55 - protein, 7 aa, synthetic construct
QSVSSSY

SEQ ID NO: 56 - protein, 9 aa, synthetic construct
QQKPGLAPR

SEQ ID NO: 57 - protein, 17 aa, synthetic construct
LAWYQQKPGLAPRLLIY

SEQ ID NO: 58 - protein, 10 aa, synthetic construct
LLIYDASSRA

SEQ ID NO: 59 - protein, 33 aa, synthetic construct
TGIPDRFSGSGSGTDFTLTISRLEPEDFAVYYC

SEQ ID NO: 60 - protein, 37 aa, synthetic construct
SSRATGIPDRFSGSGSGTDFTLTISRLEPEDFAVYYC

SEQ ID NO: 61 - protein, 7 aa, synthetic construct
QQYGSSL

SEQ ID NO: 62 - protein, 11 aa, synthetic construct
TFGQGTKVEIK

SEQ ID NO: 63 - protein, 41 aa, synthetic construct
TNYNPSLKSRVTISVDKSKNHFSLYVSSVTAADTAVYYCAR

SEQ ID NO: 64 - protein, 39 aa, synthetic construct
YNPSLKSRVTISVDKSKNHFSLYVSSVTAADTAVYYCAR

SEQ ID NO: 65 - protein, 37 aa, synthetic construct
YNPSLKSRVTISVDKSKNHFSLYVSSVTAADTAVYYC

SEQ ID NO: 66 - protein, 38 aa, synthetic construct
NYNPSLKSRVTISVDKSKNHFSLYVSSVTAADTAVYYC

SEQ ID NO: 67 - protein, 8 aa, synthetic construct
ARARLHFD

SEQ ID NO: 68 - protein, 9 aa, synthetic construct
ARARLHFDY

SEQ ID NO: 69 - protein, 12 aa, synthetic construct
YWGQGTLVTVSS

SEQ ID NO: 70 - protein, 29 aa, synthetic construct
DIVMTQSPLSLPVTPGEPASISCRSSQSL

SEQ ID NO: 71 - protein, 26 aa, synthetic construct
DIVMTQSPLSLPVTPGEPASISCRSS

SEQ ID NO: 72 - protein, 12 aa, synthetic construct
LHSNGYNYLDWY

SEQ ID NO: 73 - protein, 11 aa, synthetic construct
QSLLHSNGYNY

SEQ ID NO: 74 - protein, 9 aa, synthetic construct
LQKPGQSPQ

SEQ ID NO: 75 - protein, 17 aa, synthetic construct
LDWYLQKPGQSPQLLIY

SEQ ID NO: 76 - protein, 10 aa, synthetic construct
LLIYLGSNRA

SEQ ID NO: 77 - protein, 33 aa, synthetic construct
SGVPDRFSGSGSGTDFTLKISRVEAEDVGVYYC

SEQ ID NO: 78 - protein, 37 aa, synthetic construct
SNRASGVPDRFSGSGSGTDFTLKISRVEAEDVGVYYC

SEQ ID NO: 79 - protein, 10 aa, synthetic construct
MQALQTPPRF

SEQ ID NO: 80 - protein, 11 aa, synthetic construct
TFGPGTKVDIK

SEQ ID NO: 81 - protein, 41 aa, synthetic construct
TNYNPSLKSRVTISVDTSKNHFYLNLSSVTAADTALYYCAR

SEQ ID NO: 82 - protein, 39 aa, synthetic construct
YNPSLKSRVTISVDTSKNHFYLNLSSVTAADTALYYCAR

SEQ ID NO: 83 - protein, 37 aa, Synthetic construct
YNPSLKSRVTISVDTSKNHFYLNLSSVTAADTALYYC

SEQ ID NO: 84 - protein, 38 aa, synthetic construct
NYNPSLKSRVTISVDTSKNHFYLNLSSVTAADTALYYC

SEQ ID NO: 85 - protein, 10 aa, synthetic construct
ARSYFDSGMD

SEQ ID NO: 86 - protein, 11 aa, synthetic construct
ARSYFDSGMDV

SEQ ID NO: 87 - protein, 26 aa, synthetic construct
EIVMTQSPATLSVSPGERATLSCRAS

SEQ ID NO: 88 - protein, 6 aa, synthetic construct
QSVSSN

SEQ ID NO: 89 - protein, 17 aa, synthetic construct
LAWYQQKLGQASRLLIY

SEQ ID NO: 90 - protein, 126 aa, synthetic construct
QVQLQESGPGLVKPPGTLSLTCAVSGGSISSSNWWSWVRQPPGKGLEWIGEIYHSGSTNYNPSLKSRVTISVDTSKNQISLQLSSVTAADTAVYYCARDKMVRGLIDYYYYGLDVWGQGTTVTVSS

SEQ ID NO: 91 - protein, 116 aa, synthetic construct
QVQLQESGPGLVKPPGTLSLTCAVSGGSISSSNWWSWVRQPPGKGLEWIGEIYHSGSTNYNPSLKSRVTISVDKSKNHFSLYVSSVTAADTAVYYCARARLHFDYWGQGTLVTVSS

SEQ ID NO: 92 - protein, 118 aa, synthetic construct
QVQLQESGPGLVKPPGTLSLTCAVSGGSISSSNWWSWVRQPPGKGLEWIGEIYHSGSTNYNPSLKSRVTISVDTSKNHFYLNLSSVTAADTALYYCARSYFDSGMDVWGQGTTVTVSS

SEQ ID NO: 93 - protein, 107 aa, synthetic construct
EIVLTQSPATLSLSPGERATLSCGASQSVSSSYLAWYQQKPGLAPRLLIYDASSRATGIPDRFSGSGSGTDFTLTISRLEPEDFAVYYCQQYGSSLTFGQGTKVEIK

SEQ ID NO: 94 - protein, 114 aa, synthetic construct
DIVMTQSPLSLPVTPGEPASISCRSSQSLLHSNGYNYLDWYLQKPGQSPQLLIYLGSNRASGVPDRFSGSGSGTDFTLKISRVEAEDVGVYYCMQALQTPPRFTFGPGTKVDIK

SEQ ID NO: 95 - protein, 96 aa, synthetic construct
EIVMTQSPATLSVSPGERATLSCRASQSVSSNLAWYQQKLGQASRLLIYGASGSGSGTEFTLTISSLQSEDFAVYYCQQYNKWPVTFGQGTKLEIK

SEQ ID NO: 96 - DNA, 379 bp, synthetic construct
  source 1..379: mol_type = other DNA
caggtgcagctgcaggagtcgggcccaggactggtgaagcctccggggaccctgtccctcacctgcgctgtctctggtggctccatcagcagtagtaactggtggagttgggtccgccagcccccagggaaggggctggagtggattggggaaatctatcatagtgggagcaccaactacaacccgtccctcaagagtcgagtcaccatatcagtagacacgtccaagaaccagatctccctgcagctgagctccgtgaccgctgcggacacggccgtgtattactgtgcgagagataagatggttcggggacttattgactactactactacggtttggacgtctgggggcaagggaccacggtcaccgtctcctcag

SEQ ID NO: 97 - DNA, 349 bp, synthetic construct
  source 1..349: mol_type = other DNA
caggtgcagctgcaggagtcgggcccaggactggtgaagcctccggggaccctgtccctcacctgcgctgtctctggtggctccatcagcagtagtaactggtggagttgggtccgccagcccccagggaaggggctggagtggattggggaaatctatcatagtgggagcaccaactacaacccgtccctcaagagtcgagtcaccatatcagtagacaagtccaagaaccacttctccctgtacgtgagctctgtgaccgccgcggacacggccgtgtattactgtgcgagagcgagactacactttgactactggggccaaggaaccctggtcaccgtctcctcag

SEQ ID NO: 98 - DNA, 355 bp, synthetic construct
  source 1..355: mol_type = other DNA
caggtgcagctgcaggagtcgggcccaggactggtgaagcctccggggaccctgtccctcacctgcgctgtctctggtggctccatcagcagtagtaactggtggagttgggtccgccagcccccagggaaggggctggagtggattggggaaatctatcatagtgggagcaccaactacaacccgtccctcaagagtcgagtcaccatatcagtagacacgtccaagaaccacttctacctgaacctgagctctgtgaccgctgcggacacggccctgtattactgtgcgagaagctattttgacagcggtatggacgtctgggggcaagggaccacggtcaccgtctcctcag

SEQ ID NO: 99 - DNA, 322 bp, synthetic construct
  source 1..322: mol_type = other DNA
gaaattgtgttgacgcagtctccagccaccctgtctttgtctccaggggaaagagccaccctctcctgcggggccagtcagagtgttagcagcagctacttagcctggtaccagcagaaacctggcctggcgcccaggctcctcatctatgatgcatccagcagggccactggcatcccagacaggttcagtggcagtgggtctgggacagacttcactctcaccatcagcagactggagcctgaagattttgcagtgtattactgtcagcagtatggtagctccctcacgttcggccaagggaccaaggtggaaatcaaac

SEQ ID NO: 100 - DNA, 343 bp, synthetic construct
  source 1..343: mol_type = other DNA
gatattgtgatgactcagtctccactctccctgcccgtcacccctggagagccggcctccatctcctgcaggtctagtcagagcctcctgcatagtaatggatacaactatttggattggtacctgcagaagccagggcagtctccacagctcctgatctatttgggttctaatcgggcctccggggtccctgacaggttcagtggcagtggatcaggcacagattttacactgaaaatcagcagagtggaggctgaggatgttggggtttattactgcatgcaagctctacaaactcccccgagattcactttcggccctgggaccaaagtggatatcaaac

SEQ ID NO: 101 - DNA, 289 bp, synthetic construct
  source 1..289: mol_type = other DNA
gaaatagtgatgacgcagtctccagccaccctgtctgtgtctccaggggaaagagccaccctctcctgcagggccagtcagagtgttagtagcaacttagcctggtaccagcagaaacttggccaggcttccaggctcctcatctatggtgcatcgggcagtgggtctgggacagagttcactctcaccatcagcagcctgcagtctgaagattttgcagtttattactgtcagcagtataataagtggcctgtcacttttggccaggggaccaagttggagatcaaac

SEQ ID NO: 102 - protein, 19 aa, Homo sapiens
CAKSGRYFDWRRRGEFDYW

SEQ ID NO: 103 - protein, 13 aa, Homo sapiens
CARQKTSMLIEHW

SEQ ID NO: 104 - protein, 21 aa, Homo sapiens
CARDKMVRGLIDYYYYGLDVW

SEQ ID NO: 105 - protein, 11 aa, Homo sapiens
CARARLHFDYW

SEQ ID NO: 106 - protein, 14 aa, Homo sapiens
CAKSLMVRGVSDYW

SEQ ID NO: 107 - protein, 12 aa, Homo sapiens
CQTWDISTFVVF

SEQ ID NO: 108 - protein, 12 aa, Homo sapiens [sequence omitted]

SEQ ID NO: 109 - protein, 12 aa, Homo sapiens
CSSYSGSINFVF

SEQ ID NO: 110 - protein, 11 aa, Homo sapiens [sequence omitted]

SEQ ID NO: 111 - protein, 12 aa, Homo sapiens [sequence omitted]

SEQ ID NO: 112 - protein, 11 aa, Homo sapiens
CQHSSSYPWTF

SEQ ID NO: 113 - protein, 11 aa, Homo sapiens [sequence omitted]

SEQ ID NO: 114 - protein, 10 aa, Homo sapiens [sequence omitted]

SEQ ID NO: 115 - protein, 13 aa, Homo sapiens [sequence omitted]

SEQ ID NO: 116 - protein, 10 aa, Homo sapiens [sequence omitted]

SEQ ID NO: 117 - protein, 14 aa, Homo sapiens
CARLPPYPKDFDYW

SEQ ID NO: 118 - protein, 15 aa, Homo sapiens
CARHSSSGYYWIDYW

SEQ ID NO: 119 - protein, 19 aa, Homo sapiens
CARLMRSGILTGYYYFDYW

SEQ ID NO: 120 - protein, 15 aa, Homo sapiens
CARLDIAGRSAFDIW

SEQ ID NO: 121 - protein, 29 aa, Homo sapiens
CARIRGGVAFCGGDCEGDYFDYWDYFDYW

SEQ ID NO: 122 - protein, 12 aa, Homo sapiens
CMEALHTPPYTF

SEQ ID NO: 123 - protein, 12 aa, Homo sapiens [sequence omitted]

SEQ ID NO: 124 - protein, 12 aa, Homo sapiens
CMQCLHTPPYTF

SEQ ID NO: 125 - protein, 12 aa, Homo sapiens
CMEALQTPPFTF

SEQ ID NO: 126 - protein, 11 aa, Homo sapiens [sequence omitted]

SEQ ID NO: 127 - protein, 14 aa, Homo sapiens
CATWDDGLEGLVVF

SEQ ID NO: 128 - protein, 13 aa, Homo sapiens [sequence omitted]

SEQ ID NO: 129 - protein, 14 aa, Homo sapiens [sequence omitted]

SEQ ID NO: 130 - protein, 11 aa, Homo sapiens [sequence omitted]

SEQ ID NO: 131 - protein, 12 aa, Homo sapiens [sequence omitted]

SEQ ID NO: 132 - protein, 13 aa, Homo sapiens
CASCSTVTTFDYW

SEQ ID NO: 133 - protein, 16 aa, Homo sapiens
CAREDYGEGFDAFDIW

SEQ ID NO: 134 - protein, 13 aa, Homo sapiens
CARSYFDSGMDVW

SEQ ID NO: 135 - protein, 22 aa, Homo sapiens
CARAPSYDFWSGYYSQGAFDIW

SEQ ID NO: 136 - protein, 13 aa, Homo sapiens
CARGYGGYVLFYW

SEQ ID NO: 137 - protein, 11 aa, Homo sapiens [sequence omitted]

SEQ ID NO: 138 - protein, 12 aa, Homo sapiens
CMQSLQTPPVTF

SEQ ID NO: 139 - protein, 11 aa, Homo sapiens [sequence omitted]

SEQ ID NO: 140 - protein, 11 aa, Homo sapiens [sequence omitted]

SEQ ID NO: 141 - protein, 12 aa, Homo sapiens [sequence omitted]

SEQ ID NO: 142 - protein, 12 aa, Homo sapiens [sequence omitted]

SEQ ID NO: 143 - protein, 11 aa, Homo sapiens [sequence omitted]

SEQ ID NO: 144 - protein, 12 aa, Homo sapiens [sequence omitted]

SEQ ID NO: 145 - protein, 13 aa, Homo sapiens
CTSYRSTTVSYVF

SEQ ID NO: 146 - protein, 12 aa, Homo sapiens [sequence omitted]

SEQ ID NO: 147 - protein, 14 aa, Homo sapiens
CAREEGTSVAFDIW

SEQ ID NO: 148 - protein, 20 aa, Homo sapiens
CARERMYFYDTIGYSPFDSW

SEQ ID NO: 149 - protein, 11 aa, Homo sapiens [sequence omitted]

SEQ ID NO: 150 - protein, 11 aa, Homo sapiens [sequence omitted]

SEQ ID NO: 151 - protein, 12 aa, Homo sapiens [sequence omitted]

SEQ ID NO: 152 - protein, 13 aa, Homo sapiens
CAAWDDTLHGVVF

SEQ ID NO: 153 - protein, 20 aa, Homo sapiens
CAREGAGDGYNPIPRYFDLW

SEQ ID NO: 154 - protein, 20 aa, Homo sapiens
CARAGVLGLTQGVNRAFDIW

SEQ ID NO: 155 - protein, 13 aa, Homo sapiens
CQQLNSYPRALTF

SEQ ID NO: 156 - protein, 11 aa, Homo sapiens [sequence omitted]

SEQ ID NO: 157 - protein, 15 aa, Homo sapiens [sequence omitted]

SEQ ID NO: 158 - protein, 12 aa, Homo sapiens [sequence omitted]